European Patent Application EP 4 397 763 A1, published July 10, 2024. Title: Microorganism having improved protein productivity and their use. Applicant: AMANO ENZYME INC. The sequence listing filed with the application follows.

SEQUENCE LISTING (2 sequences)

SEQ ID NO: 1 - DNA, 738 bp, Bacillus amyloliquefaciens
  source 1..738: mol_type = genomic DNA
  CDS 1..738
atgcacgcgattgagctgaagcaattaactaaacattataaagaaaccgccgctgttgaccgacttgaattttcaattgaaaaaggagaatttttcgctttactcggagagaacggagccggaaaaacgacattaatccggatgctttgcggcctcctttctccagatgaaggtgatgcatcagtgcttggtcacagcattttgactgatttggataaaataaaaccgaaaatgaatatgtctccgcaggaaacagccatcgcccctaatttaaccgtacgggaaaacttagagtttatagccggagtctacggaattccgaaaaaagaaggaaaaaaaagaacggatgagatgctcgaattgtttcaattaaaagaaaaagaaagagaaaaaacaaaaacgttatcaggcggaatgcagcgccggctcagcatcgcaatgggaatgattacaaaaccggatatttatttcttagatgagccgacattaggtctggacgtccgttcacgccgcgagttgtggaaaaatcttgagtcattaaagggagacatgacgatcattttaacgacacactatctagaagaagctgaagccctggcagaccgtatttgcattttagaaaatgggacattaaaagcactgggtacggctgaggacctgaaaaagcaaactcattcagccacatttgaagatgcctttttagcgatttgtgacggggaggcggggctttatgcttga

SEQ ID NO: 2 - protein, 245 aa, Bacillus amyloliquefaciens
MHAIELKQLTKHYKETAAVDRLEFSIEKGEFFALLGENGAGKTTLIRMLCGLLSPDEGDASVLGHSILTDLDKIKPKMNMSPQETAIAPNLTVRENLEFIAGVYGIPKKEGKKRTDEMLELFQLKEKEREKTKTLSGGMQRRLSIAMGMITKPDIYFLDEPTLGLDVRSRRELWKNLESLKGDMTIILTTHYLEEAEALADRICILENGTLKALGTAEDLKKQTHSATFEDAFLAICDGEAGLYA